European Patent Application EP 4 379 060 A1, published June 5, 2024. Title: High-efficiency production of hydroxyectoine. Applicant: Universität des Saarlandes. The sequence listing filed with the application follows.

SEQUENCE LISTING (78 sequences)

SEQ ID NO: 1 - DNA, 6340 bp, synthetic construct
  source 1..6340: mol_type = other DNA
gatctttgggagcagtccttgtgcgcttacgaggtgagccggtggggaaccgttatctgcctatggtgtgagcccccctagagagcttcaagagcaatcagcccgacctagaaaggaggccaagagagagacccctacggggggaaccgttttctgcctacgagatggcacatttactgggaagctttacggcgtcctcgtggaagttcaatgcccgcagacttaagtgctctattcacggtctgacgtgacacgctaaattcagacatagcttcattgattgtcgccacgagccagtctctccctcaacagtcataaaccaacctgcaatggtcaagcgatttcctttagctttcctagcttgtcgttgactggacttagctagtttttctcgctgtgctcgggcgtactcactgtttgggtctttccagcgttctgcggcctttttaccgccacgtcttcccatagtggccagagcttttcgccctcggctgctctgcgtctctgtctgacgagcagggacgactggctggcctttagcgacgtagccgcgcacacgtcgcgccatcgtctggcggtcacgcatcggcggcagatcaggctcacggccgtctgctccgaccgcctgagcgacggtgtaggcacgctcgtaggcgtcgatgatcttggtgtcttttaggcgctcaccagccgcttttaactggtatcccacagtcaaagcgtggcgaaaagccgtctcatcacgggcggcacgccctggagcagtccagaggacacggacgccgtcgatcagctctccagacgcttcagcggcgctcggcaggcttgcttcaagcgtggcaagtgcttttgcttccgcagtggcttttcttgccgcttcgatacgtgcccgtccgctagaaaactcctgctcatagcgttttttaggtttttctgtgcctgagatcatgcgagcaacctccataagatcagctaggcgatccacgcgattgtgctgggcatgccagcggtacgcggtgggatcgtcggagacgtgcagtggccaccggctcagcctatgtgaaaaagcctggtcagcgccgaaaacgcgggtcatttcctcggtcgttgcagccagcaggcgcatattcgggctgctcatgcctgctgcggcatacaccggatcaatgagccagatgagctggcatttcccgctcagtggattcacgccgatccaagctggcgctttttccaggcgtgcccagcgctccaaaatcgcgtagacctcggggtttacgtgctcgattttcccgccggcctggtggctcggcacatcaatgtccaggacaagcacggctgcgtgctgcgcgtgcgtcagagcaacatactggcaccgggcaagcgattttgaaccaactcggtataacttcggctgtgtttctcccgtgtccgggtctttgatccaagcgctggcgaagtcgcgggtcttgctgccctggaaattttctctgcccaggtgagcgaggaattcgcggcggtcttcgctcgtccagccacgtgatcgcagcgcgagctcgggatgggtgtcgaacagatcagcggaaaatttccaggccggtgtgtcaatgtctcgtgaatccgctagagtcatttttgagcgctttctcccaggtttggactgggggttagccgacgccctgtgagttaccgctcacggggcgttcaacatttttcaggtattcgtgcagcttatcgcttcttgccgcctgtgcgctttttcgacgcgcgacgctgctgccgattcggtgcaggtggtggcggcgctgacacgtcctgggcggccacggccacacgaaacgcggcatttacgatgtttgtcatgcctgcgggcaccgcgccacgatcgcggataattctcgctgccgcttccagctctgtgacgaccatggccaaaatttcgctcgggggacgcacttccagcgccatttgcgacctagccgcctccagctcctcggcgtggcgtttgttggcgcgctcgcggctggctgcggcacgacacgcatctgagcaatattttgcgcgccgtcctcgcgggtcaggccggggaggaatcaggccaccgcagtaggcgcaactgattcgatcctccactactgtgcgtcctcctggcgctgccgagcacgcagctcgtcagccagctcctcaagatccgccacgagagtttctaggtcgctcgcggcactggcccagtctcgtgatgctggcgcgtccgtcgtatcgagagctcggaaaaatccgatcaccgtttttaaatcgacggcagcatcgagcgcgtcggactccagcgcgacatcagagagatccatagctgatgattcgggccaattttggtacttcgtcgtgaaggtcatgacaccattataacgaacgttcgttaaagttttggcggaaaatcacgcggcacgaaaattttcacgaagcgggactttgcgcagctcaggggtgctaaaaattttgtatcgcacttgatttttccgaaagacagattatctgcaaacggtgtgtcgtatttctggcttggtttttaaaaaatctggaatcgaaaatttgcggggcgaccgagaagttttttacaaaaggcaaaaactttttcgggatcgacagaaataaaacgatcgacggtacgcaacaaaaaagcgtcaggatcgccgtagagcgattgaagaccgtcaaccaaaggggaagcctccaatcgacgcgacgcgcgctctacggcgatcctgacgcagatttttagctatctgtcgcagcgccctcagggacaagccacccgcacaacgtcgcgagggcgatcagcgacgccgcagtactgatcctccggcgttcagcctgtgccacagccgacaggatggtgaccgcgcaattaaccctcactaaagggaacaaaagctgggtaccgggccccccctcgaggtcgacggtacctctatctggtgccctaaacgggggaatattaacgggcccagggtggtcgcaccttggttggtaggagtagcatgggatcctctagaggcccagccggccattataattaggcctcgggggccgcggccgctgcctggcggcagtagcgcggtggtcccacctgaccccatgccgaactcagaagtgaaacgccgtagcgccgatggtagtgtggggtctccccatgcgagagtagggaactgccaggcatcaaataaaacgaaaggctcagtcgaaagactgggcctttcgttttatctgttgtttgtcggtgaacgctctcctgagtaggacaaatccgccgggagcggatttgaacgttgcgaagcaacggcccggagggtggcgggcaggacgcccgccataaactgccaggcatcaaattaagcagaaggccatcctgacggatggccttttgaagacaaggccgccaccgcggtggagctccaattcgccctatagtgagtcgtattacgcgcggtgaccaccatttgccccatatcaccgtcggtactgatcccgtcgtcaataaaccgaaccgctacaccctgagcatcaaactcttttatcagttggatcatgtcggcggtgtcgcggccaagacggtcgagcttcttcaccagaatgacatcaccttcctccaccttcatcctcagcaaatccagcccttcccgatctgttgaactgccggatgccttgtcggtaaagatgcggttagcttttacccctgcatctttgagcgctgaggtctgcctcgtgaagaaggtgttgctgactcataccaggcctgaatcgccccatcatccagccagaaagtgagggagccacggttgatgagagctttgttgtaggtggaccagttggtgattttgaacttttgctttgccacggaacggtctgcgttgtcgggaagatgcgtgatctgatccttcaactcagcaaaagttcgatttattcaacaaagccgccgtcccgtcaagtcagcgtaatgctctgccagtgttacaaccaattaaccaattctgattagaaaaactcatcgagcatcaaatgaaactgcaatttattcatatcaggattatcaataccatatttttgaaaaagccgtttctgtaatgaaggagaaaactcaccgaggcagttccataggatggcaagatcctggtatcggtctgcgattccgactcgtccaacatcaatacaacctattaatttcccctcgtcaaaaataaggttatcaagtgagaaatcaccatgagtgacgactgaatccggtgagaatggcaaaagcttatgcatttctttccagacttgttcaacaggccagccattacgctcgtcatcaaaatcactcgcatcaaccaaaccgttattcattcgtgattgcgcctgagcgagacgaaatacgcgatcgctgttaaaaggacaattacaaacaggaatcgaatgcaaccggcgcaggaacactgccagcgcatcaacaatattttcacctgaatcaggatattcttctaatacctggaatgctgttttcccggggatcgcagtggtgagtaaccatgcatcatcaggagtacggataaaatgcttgatggtcggaagaggcataaattccgtcagccagtttagtctgaccatctcatctgtaacatcattggcaacgctacctttgccatgtttcagaaacaactctggcgcatcgggcttcccatacaatcgatagattgtcgcacctgattgcccgacattatcgcgagcccatttatacccatataaatcagcatccatgttggaatttaatcgcggcctcgagcaagacgtttcccgttgaatatggctcataacaccccttgtattactgtttatgtaagcagacagttttattgttcatgatgatatatttttatcttgtgcaatgtaacatcagagattttgagacacaacgtggctttgttgaataaatcgaacttttgctgagttgaaggatcagatcacgcatcttcccgacaacgcagaccgttccgtggcaaagcaaaagttcaaaatcaccaactggtccacctacaacaaagctctcatcaaccgtggctccctcactttctggctggatgatggggcgattcaggcctggtatgagtcagcaacaccttcttcacgaggcagacctcagcgctagcggagtgtatactggcttactatgttggcactgatgagggtgtcagtgaagtgcttcatgtggcaggagaaaaaaggctgcaccggtgcgtcagcagaatatgtgatacaggatatattccgcttcctcgctcactgactcgctacgctcggtcgttcgactgcggcgagcggaaatggcttacgaacggggcggagatttcctggaagatgccaggaagatacttaacagggaagtgagagggccgcggcaaagccgtttttccataggctccgcccccctgacaagcatcacgaaatctgacgctcaaatcagtggtggcgaaacccgacaggactataaagataccaggcgtttccccctggcggctccctcgtgcgctctcctgttcctgcctttcggtttaccggtgtcattccgctgttatggccgcgtttgtctcattccacgcctgacactcagttccgggtaggcagttcgctccaagctggactgtatgcacgaaccccccgttcagtccgaccgctgcgccttatccggtaactatcgtcttgagtccaacccggaaagacatgcaaaagcaccactggcagcagccactggtaattgatttagaggagttagtcttgaagtcatgcgccggttaaggctaaactgaaaggacaagttttggtgactgcgctcctccaagccagttacctcggttcaaagagttggtagctcagagaaccttcgaaaaaccgccctgcaaggcggttttttcgttttcagagcaagagattacgcgcagaccaaaacgatctcaagaagatcatcttattaaggggtctgacgctcagtggaacgaaaactcacgttaagggattttggtcatgagattatcaaaaaggatcttcacctagatccttttaaattaaaaatgaagttttaaatcaatctaaagtatatatgagtaaacttggtctgacagttaccaatgcttaatcagtgaggcacctatctcagcgatctgtctatttcgttcatccatagttgcctgactccccgtcgtgtagataactacgatacgggagggcttaccatctggccccagtgctgcaatgataccgcgagacccacgctcaccggctccagatttatcagcaataaaccagccagccg

SEQ ID NO: 2 - DNA, 5106 bp, synthetic construct
  source 1..5106: mol_type = other DNA
tcgatttaaatctcgagaggcctgacgtcgggcccggtaccacgcgtcatatgactagttcggacctagggatatcgtcgacatcgatgctcttctgcgttaattaacaattgggatcctctagacccgggatttaaatgatccgctagcgggctgctaaaggaagcggaacacgtagaaagccagtccgcagaacggtgctgacccggatgaatgtcagctactgggctatctggacagggaaaacgcaagcgcaaagagaaagcaggtagcttgcagtgggcttacatggcgatagctagactgggcggttttatggacagcaagcgaaccggaattgccagctggggcgccctctggtaaggttgggaagccctgcaaagtaaactggatggctttcttgccgccaaggatctgatggcgcaggggatcaagatctgatcaagagacaggatgaggatcgtttcgcatgattgaacaagatggattgcacgcaggttctccggccgcttgggtggagaggctattcggctatgactgggcacaacagacaatcggctgctctgatgccgccgtgttccggctgtcagcgcaggggcgcccggttctttttgtcaagaccgacctgtccggtgccctgaatgaactgcaggacgaggcagcgcggctatcgtggctggccacgacgggcgttccttgcgcagctgtgctcgacgttgtcactgaagcgggaagggactggctgctattgggcgaagtgccggggcaggatctcctgtcatctcaccttgctcctgccgagaaagtatccatcatggctgatgcaatgcggcggctgcatacgcttgatccggctacctgcccattcgaccaccaagcgaaacatcgcatcgagcgagcacgtactcggatggaagccggtcttgtcgatcaggatgatctggacgaagagcatcaggggctcgcgccagccgaactgttcgccaggctcaaggcgcgcatgcccgacggcgaggatctcgtcgtgacccatggcgatgcctgcttgccgaatatcatggtggaaaatggccgcttttctggattcatcgactgtggccggctgggtgtggcggaccgctatcaggacatagcgttggctacccgtgatattgctgaagagcttggcggcgaatgggctgaccgcttcctcgtgctttacggtatcgccgctcccgattcgcagcgcatcgccttctatcgccttcttgacgagttcttctgagcgggactctggggttcgaaatgaccgaccaagcgacgcccaacctgccatcacgagatttcgattccaccgccgccttctatgaaaggttgggcttcggaatcgttttccgggacgccggctggatgatcctccagcgcggggatctcatgctggagttcttcgcccacgctagcggcgcgccggccggcccggtgtgaaataccgcacagatgcgtaaggagaaaataccgcatcaggcgctcttccgcttcctcgctcactgactcgctgcgctcggtcgttcggctgcggcgagcggtatcagctcactcaaaggcggtaatacggttatccacagaatcaggggataacgcaggaaagaacatgtgagcaaaaggccagcaaaaggccaggaaccgtaaaaaggccgcgttgctggcgtttttccataggctccgcccccctgacgagcatcacaaaaatcgacgctcaagtcagaggtggcgaaacccgacaggactataaagataccaggcgtttccccctggaagctccctcgtgcgctctcctgttccgaccctgccgcttaccggatacctgtccgcctttctcccttcgggaagcgtggcgctttctcatagctcacgctgtaggtatctcagttcggtgtaggtcgttcgctccaagctgggctgtgtgcacgaaccccccgttcagcccgaccgctgcgccttatccggtaactatcgtcttgagtccaacccggtaagacacgacttatcgccactggcagcagccactggtaacaggattagcagagcgaggtatgtaggcggtgctacagagttcttgaagtggtggcctaactacggctacactagaaggacagtatttggtatctgcgctctgctgaagccagttaccttcggaaaaagagttggtagctcttgatccggcaaacaaaccaccgctggtagcggtggtttttttgtttgcaagcagcagattacgcgcagaaaaaaaggatctcaagaagatcctttgatcttttctacggggtctgacgctcagtggaacgaaaactcacgttaagggattttggtcatgagattatcaaaaaggatcttcacctagatccttttaaaggccggccgcggccgcgcaaagtcccgcttcgtgaaaattttcgtgccgcgtgattttccgccaaaaactttaacgaacgttcgttataatggtgtcatgaccttcacgacgaagtaccaaaattggcccgaatcatcagctatggatctctctgatgtcgcgctggagtccgacgcgctcgatgctgccgtcgatttaaaaacggtgatcggatttttccgagctctcgatacgacggacgcgccagcatcacgagactgggccagtgccgcgagcgacctagaaactctcgtggcggatcttgaggagctggctgacgagctgcgtgctcggcagcgccaggaggacgcacagtagtggaggatcgaatcagttgcgcctactgcggtggcctgattcctccccggcctgacccgcgaggacggcgcgcaaaatattgctcagatgcgtgtcgtgccgcagccagccgcgagcgcgccaacaaacgccacgccgaggagctggaggcggctaggtcgcaaatggcgctggaagtgcgtcccccgagcgaaattttggccatggtcgtcacagagctggaagcggcagcgagaattatccgcgatcgtggcgcggtgcccgcaggcatgacaaacatcgtaaatgccgcgtttcgtgtggccgtggccgcccaggacgtgtcagcgccgccaccacttgcaccgaatcggcagcagcgtcgcgcgtcgaaaaagcgcacaggcggcaagaagcgataagctgcacgaatacctgaaaaatgttgaacgccccgtgagcggtaactcacagggcgtcggctaacccccagtccaaacctgggagaaagcgctcaaaaatgactctagcggattcacgagacattgacacaccggcctggaaattttccgctgatctgttcgacacccatcccgagctcgcgctgcgatcacgtggctggacgagcgaagaccgccgcgaattcctcgctcacctgggcagagaaaatttccagggcagcaagacccgcgacttcgccagcgcttggatcaaagacccggacacgggagaaacacagccgaagttataccgagttggttcaaaatcgcttgcccggtgccagtatgttgctctgacgcacgcgcagcacgcagccgtgcttgtcctggacattgatgtgccgagccaccaggccggcgggaaaatcgagcacgtaaaccccgaggtctacgcgattttggagcgctgggcacgcctggaaaaagcgccagcttggatcggcgtgaatccactgaagcgggaaatgccagctcatctggctcattgatccggtgtatgccgcagcaggcatgagcagcccgaatatgcgcctgctggctgcaacgaccgaggaaatgacccgcgttttcggcgctgaccaggctttttcacataggctgagccggtggccactgcacgtctccgacgatcccaccgcgtaccgctggcatgcccagcacaatcgcgtggatcgcctagctgatcttatggaggttgctcgcatgatctcaggcacagaaaaacctaaaaaacgctatgagcaggagttttctagcggacgggcacgtatcgaagcggcaagaaaagccactgcggaagcaaaagcacttgccacgcttgaagcaagcctgccgagcgccgctgaagcgtctggagagctgatcgacggcgtccgtgtcctctggactgctccagggcgtgccgcccgtgatgagacggcttttcgccacgctttgactgtgggataccagttaaaagcggctggtgagcgcctaaaagacaccaagatcatcgacgcctacgagcgtgcctacaccgtcgctcaggcggtcggagcagacggccgtgagcctgatctgccgccgatgctgtgaccgccagacgatggcgcgacgtgtgcgcggctacgtcgctaaaggccagccagtcgtccctgctcgtcagacagagacgcagagcagccgagggcgaaaagctctggccactatgggaagacgtggcggtaaaaaggccgcagaacgctggaaagacccaaacagtgagtacgcccgagcacagcgagaaaaactagctaagtccagtcaacgacaagctaggaaagctaaaggaaatcgcttgaccattgcaggttggtttatgactgttgagggagagactggctcgtggccgacaatcaatgaagctatgtctgaatttagcgtgtcacgtcagaccgtgaatagagcacttaagtctgcgggcattgaacttccacgaggacgccgtaaagcttcccagtaaatgtgccatctcgtaggcagaaaacggttccccccgtaggggtctctctcttggcctcctttctaggtcgggctgattgctcttgaagctctctaggggggctcacaccataggcagataacggttccccaccggctcacctcgtaagcgcacaaggactgctcccaaagatcttcaaagccactgccgcgactccgcttcgcgaagccttgccccgcggaaatttcctccaccgagttcgtgcacacccctatgccaagcttctttcaccctaaattcgagagattggattcttaccgtggaaattcttcgcaaaaatcgtcccctgatcgcccttgcgacgttgctcgcggtcggtgccgctggttgcgcttggcttgaccgacttgagcggccgc

SEQ ID NO: 3 - DNA, 200 bp, synthetic construct
  source 1..200: mol_type = other DNA
tggccgttaccctgcgaatgtccacagggtagctggtagtttgaaaatcaacgccgttgcccttaggattcagtaactggcacattttgtaatgcgctagatctgtgtgctcagtcttccaggctgcttatcacagtgaaagcaaaaccaattcgtggctgcgaaagtcgtagccaccacgaagtccaggaggacataca

SEQ ID NO: 4 - DNA, 582 bp, synthetic construct
  source 1..582: mol_type = other DNA
atgccaaccctgaagcgcaactccatcaacaacccaaagggcatcgtgctgtccttcccaaccgtgatgctgcgtcgcccaaccgatggcgacggctacaacctgcaccagctcgtggcacgctgccagccactggataccaactccgtgtactgcaacctgctgcagtgctccgatttcgcagataccgcaatcgcagcagaaaacgcacagggcgaactggtgggcttcatctccggctaccgtccaccatcccgtccagataccctgttcgtgtggcaggtcgcagtggattcctccatgcgtggccagggcctggcactgcgcatgctgctggcactgaccgcacgcgtggcacgcgaatacggcgtgcgctacatggaaaccaccatctccccagataacggtgcatcccaggcactgttcaaacgcgcattcgatcgcctggatgcaaactgcaccacccgcaccctgttcgcacgcgatacccacttcgcaggccagcacgaagatgaagtgctgtaccgtgcaggcccattcaccgtgtcccacctggaagaagaactgaaagaacacgcataa

SEQ ID NO: 5 - DNA, 1278 bp, synthetic construct
  source 1..1278: mol_type = other DNA
atgaaaaccttcgaactgaacgaatcccgtgtgcgctcctactgccgctccttcccagtggtgttcaagcaggcacagggtgcagaactggtgacccaggatggcaagcgctacatcgatttcttggcaggcgcaggcaccctgaactacggccacaaccacccagtgctgaagcaggcactgctggaatacatcgaatccgatggcatcacccacggcctggatatgtacaccgaagcaaaagaacgcttcctggaaaccttcaaccgcctgatcctggaaccacgcggtatgggcgattaccgcatgcagttcaccggtccaaccggcaccaacgcagtggaagcagcaatgaagctggcacgcaaggtgaccggtcgcaacaacatcatttccttcaccaacggcttccacggctgctccatcggtgcactggcagcaaccggcaaccagcaccaccgtggcggttccggcatcggcctgaccgatgtgtcccgcatgccatacgcaaactacttcggcgataagaccaacaccatcggcatgatggataagctgctgtccgatccatcctccggcatcgataagccagcagcagtgatcgtggaagtggtgcagggcgaaggcggtctgaacaccgcatccgcagaatggatgcgcaagctggaaaagctgtgccgcaagcacgaaatgctgctgatcgtggatgatatccaggcaggctgcggtcgtaccggtaccttcttctccttcgaagaaatgggcatccagccagatatcgtgaccctgtccaagtccctgtccggctacggcctgccattcgcaatggtgctgctgcgccaagaactggatcagtggaagccaggcgaacacaacggcaccttccgtggcaacaaccacgcattcgtgaccgcagcagcagcagtggaacacttctggcagaacgatgcattcgcaaactccgtgaaggcaaagggcaagcgcattgcagatggcatgcagcgcatcatccgtcgccacggtccagactccctgttcctgaagggtcgcggtatgatgatcggcatctcctgcccagatggcgaaatcgcagcagccgtgtgtcgccacgcattcgaaaacggcctggtgatcgaaacctccggtgcacactccgaagtggtgaagtgcctgtgcccactgatcatctccgatgagcagatcgatcaggcactgtccatcctggataaggcattcgcagcagtgatgtccgaacagaccgaaaaccaggcatcctaa

SEQ ID NO: 6 - DNA, 402 bp, synthetic construct
  source 1..402: mol_type = other DNA
atgatcgtgcgcaccctggcagaatgcgaaaagaccgatcgcaaggtgcactcccagaccggcacctgggattccacccgcatgctgctcaaggatgataaggtgggcttctccttccacatcaccaccatctacgcaggctccgaaacccacatccactaccagaaccacttcgaatccgtctactgcatctccggcaacggcgaaatcgaaaccattgccgatggcaagatctacaagatcgaaccaggcaccctgtacgtgctggaaaagcacgatgaacacctgttgcgtggtggctccgaagatatgaagctggcctgcgtgttcaacccaccactgaacggtcgcgaagtgcacgatgaatccggtgtgtacccactggaagcagaaaccgtgtaa

SEQ ID NO: 7 - DNA, 909 bp, Pseudomonas stutzeri
  source 1..909: mol_type = unassigned DNA
atgcaagccgacctgtatccctcgcgccaggaagaccagcccagctggcaggaacgcctggatccggtcgtctaccgcagcgacctggagaatgcgccgatcgcggcagagctggtcgaacgcttcgaacgcgacggctacctggtcatccccaatctgttcagcgccgacgaagtcgcgctgtttcgcgccgaactcgagcgcatgcgccaggacccggccgtcgccggttccggcaagaccatcaaggaacccgacagcggtgcgatccgctcggtgttcgccatccacaaggacaacgagctgttcgcccgcgtcgcagccgacgagcgcaccgccggcatcgcccgcttcatccttggcggcgacctgtacgtgcatcagtcgcgaatgaacttcaagcccggcttcaccggcaaggagttctactggcactcggatttcgagacctggcacatcgaggacggcatgccgcgcatgcgctgcctgtcctgctcgatcctcttgaccgacaacgagccgcacaacggcccgctgatgctgatgcccggctcgcacaagcactacgtgcgctgcgtcggagccacaccggaaaatcactacgagaagtccctgcgcaagcaggagatcggcatccccgaccagaacagcctgagcgagctggccagccgcttcggcatcgactgcgccaccggccccgccggcagcgtggtgttcttcgactgcaacaccatgcacggctccaacggcaacatcacgcccagcgcgcgtagcaatctgttctacgtctacaaccacgtggataatgccgtgcaggctccgttctgcgagcagaaaccgcgcccggcctttgtcgccgaacgcgagaatttcaagccgctggacattcggccgcaacagtatctctga

SEQ ID NO: 8 - DNA, 909 bp, synthetic construct
  source 1..909: mol_type = other DNA
atgcaggcagatctgtacccatcccgtcaagaagatcagccatcctggcaagaacgcctggatccagtggtgtaccgctccgatctggaaaacgcaccaatcgcagccgaactggtggaacgcttcgaacgcgacggctacctggtgatcccaaacctgttctccgcagatgaagtggcactgtttcgcgcagaactggaacgcatgcgccaggatccagcagtggcaggctccggcaagaccatcaaagaaccagattccggtgcaatccgctccgtgttcgcaatccacaaggataacgaactgttcgctcgcgtggcagcagatgaacgcaccgcaggtatcgcacgcttcatcctgggtggcgatctgtacgtgcaccagtcccgcatgaacttcaagccaggcttcaccggcaaagaattctactggcactccgatttcgaaacctggcacatcgaagatggcatgccacgcatgcgctgcctgtcctgctccatcctgctgaccgataacgaaccacacaacggtccactgatgctgatgccaggctcccacaagcactacgtgcgctgcgttggcgcaaccccagaaaaccactacgaaaagtccctgcgcaagcaagaaatcggcatccctgatcagaactccctgtccgaactggcatcccgcttcggcatcgattgcgcaaccggtccagcaggctccgtggtgttcttcgattgcaacaccatgcacggctccaacggcaacatcaccccatccgcacgctccaacctgttctacgtgtacaaccacgtggataacgcagtgcaggcaccattctgcgaacagaagccacgcccagcattcgtggccgaacgcgaaaacttcaagcctctggatattcgcccacagcagtacctgtaa

SEQ ID NO: 9 - DNA, 918 bp, Mycobacterium smegmatis
  source 1..918: mol_type = unassigned DNA
atgaccaccacgcagttcacccagacgacaccaaccgccgagacgcgccacgacccgtacccgacgcgcctgtcccacgcgatcgaaccgatcccgcgtgccgaccccacggtgtggggcagcgaggccgacggcccgctcaaccagaagaacctggaccacttctcgtcgcagggctacctggtgcgccacggcaccgtcaccaacgactggctgccgcacctgcgccaggaaatggaccgcatcgccgccgatctcgacgacgacgatccgcgcgtgatccgcgagccgggcgggtcgatccgctcgatcttcgaaccgcacctgctcagcgaccttgtcgcgcaggtggtccggctcgacaccgtcctgccggtggcacgccagctgctcggtagcgacgtctacatccaccaggcgcggatcaacatgatgcccgggttcaccgggacgggtttctactggcactcggatttcgagacgtggcacgccgaggacggcatgccggccatccgggccgtgtcgtgttcgatcgcgctgacccgcaactacccgtacaacgggtcgctgatggtgatccccggctcgcaccagacgttctatccgtgcgtgggggagaccccgcaggacaaccacgacacgtcgctggtggcccagacggtcggcgtccccgacgagacgacgctgaccaaggccgtcgaccacgccggcatcgatcagttcacgggagccgccgggtcggcgctgtggttcgacgccaacctgctgcacgggtccgggtccaacatcacaccgcttccgcggtccaatgtgttcctggttttcaactcggtcgacaacgcgctcgaggagcctttcgcggcgccacgacgcaggccggaatacctggcagcccgtcgggtcgcacccgtcacatag

SEQ ID NO: 10 - DNA, 918 bp, synthetic construct
  source 1..918: mol_type = other DNA
atgaccaccacccagttcacccagaccaccccaaccgcagaaaccaggcacgatccatacccaacccgcctgtcccacgcaatcgaaccaatcccacgcgcagacccaaccgtgtggggctccgaagccgatggcccactgaaccagaagaacctggaccacttctcctcccagggctacctggtgcgccacggcaccgtgaccaacgactggctgccacacctgcgccaggaaatggaccgcatcgccgcagacctggacgacgatgatccacgcgtgatccgcgaaccaggcggctccatccgctccatcttcgaaccacacctgctgtccgatctggtggcacaggtggtgcgcctggataccgtgctgccagtggcacgccagctgctgggctccgatgtgtacatccaccaggcacgcatcaacatgatgccaggcttcaccggcaccggcttctactggcactccgacttcgaaacctggcacgcagaagacggcatgccagcaatccgcgccgtgtcctgctccatcgcactgacccgcaactacccatacaacggctccctgatggtgatcccaggctcccaccagaccttctacccatgcgtgggcgaaactcctcaggataaccacgatacctccctggtggcccagaccgtgggcgtgccagatgaaaccaccctgaccaaggcagtggaccacgcaggcatcgatcagttcaccggcgcagcaggctccgcactgtggttcgatgccaacctgctgcacggctccggctccaacatcaccccactgccacgctccaacgtgttcctggtgttcaactccgtggacaacgcactggaagaaccattcgccgcaccacgccgccgcccagaatacctggcagcacgccgcgtggccccagtgacttaa

SEQ ID NO: 11 - DNA, 843 bp, Streptomyces coelicolor
  source 1..843: mol_type = unassigned DNA
gtggccacccctcggcaggacccggtcgtctggggctccccggacgcgcccggccccgtctctgcgggcgacctccaggcgctggaccgcgacggcttcctcgccatcgaccagctgatcaccccggacgaggtcggcgagtaccagcgtgagctggagcgcctcaccaccgacccggccatccgcgcggacgagcgctcgatcgtcgagccgcagtccaaggagatccggtcggtcttcgaggtgcacaagatcagtgaggtcttcgccaagctggtgcgcgacgagcgcgtggtcgggcgggcgcggcagatcctcggctcggacgtgtacgtccaccagtcgcggatcaacgtcaagccgggcttcggggccagcggtttctactggcactcggacttcgagacctggcacgccgaggacggcctgcccaacatgcgcacgatctcggtctcgatcgcgctcaccgagaactacgacaccaacggcggtctgatgatcatgccggggtcgcacaagacgttcctcgggtgcgcgggggccacgccgaaggacaactacaagaagtccctgcagatgcaggacgcggggacgccgtccgacgagggcctgacgaagatggcctcggagtacggcatcaagctgttcaccggcaaggccggttcggcgacctggttcgactgcaactgcatgcacgggtcgggcgacaacatcacgccgttcccgcgcagcaacgtgttcatcgtgttcaacagcgtggagaacacggcggtcgagccgttcgcggctccgatccggcggccggagttcatcggggcgcgggacttcacgccggtgaagtga

SEQ ID NO: 12 - DNA, 843 bp, synthetic construct
  source 1..843: mol_type = other DNA
gtggcaaccccacgccaggatccagtggtgtggggctccccagacgccccaggtccagtgtccgccggtgacctgcaggcactggaccgcgacggcttcctggcaatcgatcagctgatcaccccagacgaagtgggcgaataccagcgcgaactggaacgcctgaccaccgacccagcaatccgcgccgatgaacgctccatcgtggaaccacagtccaaggaaatccgctccgtgttcgaagtgcacaagatctccgaagtgttcgccaagctggtgcgcgatgaacgcgtggtgggccgcgcacgtcagatcctgggctccgatgtgtacgtgcaccagtcccgcatcaacgtgaagccaggcttcggcgcatccggcttctactggcactccgacttcgaaacctggcacgccgaagatggcctgccaaacatgcgcaccatctccgtgtccatcgcactgaccgaaaactacgataccaacggcggcctgatgatcatgccaggctcccacaagaccttcctgggctgcgccggcgccaccccaaaggataactacaagaagtccctgcagatgcaggatgcaggcaccccatccgatgaaggcctgaccaagatggcatccgaatacggcatcaagctgttcaccggcaaggcaggctccgccacctggttcgactgcaactgcatgcacggctccggcgacaacatcaccccattcccacgctccaacgtgttcatcgtgttcaactccgtggaaaacaccgcagtggaaccattcgcagcaccaatccgccgcccagaattcatcggcgcccgcgacttcaccccagtgaagtaa

SEQ ID NO: 13 - DNA, 927 bp, Halomonas elongata
  source 1..927: mol_type = unassigned DNA
atgtcagtgcagacatcgtccaaccgaccgctgccacaagcgaacctgcatatcgccacggagacacccgaggccgacagccggatccgtagcgcgccgcgtccggggcaggatccctatccgacccgactgagcgagccgctggatcttccctggctcaatcgccgcgagccggtggtcaagggagaggaggccgatgggccgctctcggccgcgcagctcgataccttcgagcgccagggcttcatcttcgagccggacttcctgaaaggcgaggaactcgaggcgttgcgccacgaactcaacgccctgctggcccgggatgacttccgcggacgagacttcgccatcaccgagccgcagggcaacgagatccgctcgctgttcgcggtgcactacctgtcgcgagtcttcagccgcctggccaacgacgaacgcctgatgggtcgcgcccggcagattctcggcggcgagccctatgtccatcagtcgcgcatcaactacaagcccggcttcgagggcaagggcttcaattggcattccgattttgaaacctggcacgccgaggatggcatgcccgccatgcatgcggtgagtgcgtccatcgtgctgaccgacaaccacaccttcaacgggccgctgatgctggtgcccggctcacaccgggtattcgtgccgtgcctgggtgaaacgccggaggatcatcaccggcagtcgctcaagacccaggaattcggcgtgccgagccgccaggcgctgcgcgagttgatcgaccgacatggtatcgaagcgcccaccggcgcggcgggtggcctgctgctgttcgactgcaataccctgcacggctccaacgccaacatgtcgccggatccgcgcagcaacgcctttttcgtctacaaccgtcgtgacaaccgctgcgtcgaacct

SEQ ID NO: 14 - DNA, 927 bp, synthetic construct
  source 1..927: mol_type = other DNA
atgtccgtgcagacctcctccaaccgcccactgccacaggcaaacctgcacatcgcaaccgaaactcctgaagccgattcccgcatccgctccgcaccacgcccaggtcaggacccatacccaacccgcctgtccgaaccactggacctgccatggctgaaccgccgcgaaccagtggtgaagggcgaagaagccgatggcccactgtccgcagcccagctggataccttcgaacgccagggcttcatcttcgaaccagacttcctgaagggcgaagagctggaagcactgcgccacgaactgaacgcactgctggcccgcgatgacttccgcggccgtgacttcgccatcaccgaaccacagggcaacgaaatccgctccctgttcgcagtgcactacctgtcccgcgtgttctcccgcctggcaaacgatgaacgcctgatgggccgcgcacgccagatcctgggcggtgaaccatacgtgcaccagtcccgcatcaactacaagccaggcttcgaaggcaagggcttcaactggcactccgacttcgaaacctggcacgcagaagatggcatgccagcaatgcacgccgtgtccgcatccatcgtgctgaccgacaaccacaccttcaacggcccactgatgctggtgccaggctcccaccgcgtgttcgtgccatgcctgggcgaaactcctgaggaccaccaccgccagtccctgaagacccaggaattcggcgtgccatcccgccaggcactgcgcgaactgatcgatcgccacggcatcgaagcaccaaccggcgccgccggtggcttgttgctgttcgactgcaacaccctgcacggctccaacgccaacatgtccccagatccacgctccaacgcattcttcgtgtacaaccgccgcgataaccgctgcgtggaacca

SEQ ID NO: 15 - DNA, 903 bp, Virgibacillus salexigens
  source 1..903: mol_type = unassigned DNA
atggaagatctttatccttcaagacaaaataatcaaccgaagattttgaaaaggaaggatcctgtaatctatactgatcgatccaaagataatcaagcccctattacaaaagaacagcttgattcctatgagaaaaatggatttctgcagattaaaaactttttctctgaagacgaagtgatagatatgcagaaagcgatttttgaactgcaggattcaatcaaagatgtggcttccgataaagtaatacgcgaaccggaaagcaatgacatccgttctatttttcacgttcatcaggatgataactatttccaagatgtggcaaatgacaaacgcattcttgatattgttcgtcaccttttgggaagcgatgtgtatgtacatcaatcccgaattaattataaaccgggatttaaaggaaaggagtttgactggcattctgatttcgagacatggcatgtagaagatggaatgccacggatgcgatgcatcagtgtatctattgctctatcagataactattcgtttaacggacctttgatgcttataccagggtcccataactattttgtgagttgtgtaggtgaaacacctgataataactataaagaatcattgaagaagcagaagctgggcgtacctgatgaagaaagccttcgtgaactaacaagaataggcgggggtatctctgttccaactggtaaggcaggatctgttacattgtttgaatgtaacacaatgcatggttcaaccagcaatattacaccatatccacgtaataatttattcatggtgtataatagtgttaaaaatcgtttagtggagccgttttctggtggtgaaaagcgtccggaatatatagcagtacgagagaaacaaccagtgtatagtgctgtaaactaa

SEQ ID NO: 16 - DNA, 903 bp, synthetic construct
  source 1..903: mol_type = other DNA
atggaagacctgtacccatcccgccagaacaaccagccaaagatcctgaagcgcaaggatccagtgatctacaccgaccgctccaaggataaccaggccccaatcaccaaggaacagctggactcctacgaaaagaacggcttcctgcagatcaagaacttcttctccgaagatgaagtgatcgacatgcagaaggccatcttcgaactgcaggattccatcaaggacgtggcatccgacaaggtgatccgcgaaccagaatccaacgatatccgctccatcttccacgtgcaccaggacgacaactacttccaggatgtggcaaacgacaagcgcatcctggacatcgtgcgccacctgctgggctccgatgtgtacgtgcaccagtcccgcatcaactacaagccaggcttcaagggcaaggaattcgactggcactccgacttcgaaacctggcacgtggaagacggcatgccacgcatgcgctgcatctccgtgtccatcgccctgtccgacaactactccttcaacggcccactgatgctgatcccaggctcccacaactacttcgtgtcctgcgtgggcgaaactcctgataacaactacaaggaatccctgaagaagcagaagctgggcgtgccagacgaagaatccctgcgcgaactgacccgcatcggcggcggtatctccgtgccaaccggcaaggcaggctccgtgaccctgttcgaatgcaacaccatgcacggctccacctccaacatcaccccatacccacgcaacaacctgttcatggtgtacaactccgtgaagaaccgcctggtggaaccattctccggcggcgaaaagcgcccagaatacatcgcagtgcgcgaaaagcagccagtgtactccgcagtgaactaa

SEQ ID NO: 17 - DNA, 933 bp, Gracilibacillus sp.
  source 1..933: mol_type = unassigned DNA
atgaaagatttatattcttctagaatcaaaggcatgccttctattttggaaagaaaagatccaataattcacaactcaacagcagaggatggtcctttacaacaaaaggaattagatttttacgagaaaaatggttatctatttaaacagaactttttttctaaggaagaggtaaaggtattacagcaagagttaaaacgtaatatgaatgacaatcagtcttctgatgaaccttacgtcgttagagaaactggtggcgacgaaatacgttcagtatttgatgtgcataacaacgatgaatttttccacaatttatcgtcctatgaacgtattgttgagattgcacaacatttgctaggaagtcaggtttacataaaccaatcacggattaattttaaacctggctttaaaggaaaaggcttttattggcattctgattttgaaacctggcatatggaagatggaatgcctaatatgcgtgctgttagttgcagtattattttaacggacaactattcttacaacggtccactattattaattcctggttcccatcgttactttgtacagtgtgttggggaaacacctgaaaatcattttgaacagtccttgaaaatgcaaaatatcggtgtaccagatcatgatagtattaactggttattagaaaaaggcggaagaatagacagcgctacaggaccggctgggtcagtattattctttgaatctaataccatgcatggttctaatagtaatatttcgccactgccacgtagtaatgtattttttgtctttaacagtattgaaaataaattggtggaaccattcgcggatgtttctgcaagaccagagtttgttgcaaatcgtacaaatattaaaccgatcgaaccgaaacattttaatcttaataggagaaaagtgtatttacatcaataa

SEQ ID NO: 18 - DNA, 933 bp, synthetic construct
  source 1..933: mol_type = other DNA
atgaaggatctctactcctcccgcatcaagggcatgccatccatcctggaacgcaaggacccaatcatccacaactccaccgcagaggatggcccactccagcagaaggaactggacttctacgagaagaacggctacctcttcaagcagaacttcttctccaaggaagaggtgaaggtcctccagcaggaactgaagcgcaacatgaacgataaccagtcctccgacgagccatacgtggtccgcgaaaccggcggcgatgagatccgctccgtgttcgatgtccacaacaacgacgaattcttccacaacctgtcctcctacgaacgcatcgtggagatcgcccagcacctgctcggctcccaggtctacatcaaccagtcccgcatcaacttcaagccaggcttcaagggcaagggcttctactggcactccgatttcgaaacctggcacatggaggacggcatgccaaacatgcgcgctgtgtcctgctccatcatcctgaccgacaactactcctacaacggcccactgctcctgatcccaggctcccaccgctacttcgtgcagtgcgtcggcgaaaccccagagaaccacttcgaacagtccctcaagatgcagaacatcggcgtgccagatcacgactccatcaactggctcctggaaaagggcggccgtatcgattccgcaaccggtccagctggctccgtcctgttcttcgagtccaacaccatgcacggctccaactccaacatctccccactcccacgctccaacgtgttcttcgtcttcaactccatcgaaaacaagctcgtggaaccattcgctgacgtctccgcacgcccagaattcgtggccaaccgcaccaacatcaagccaatcgagccaaagcacttcaacctcaaccgtcgcaaggtctacctgcaccagtaa

SEQ ID NO: 19 - DNA, 921 bp, Acidiphilium cryptum
  source 1..921: mol_type = unassigned DNA
atggacgatctctatccgtcgcgccgcgaacccaccccgtcgctgctgccgcgccacgatccggtggtgcatgggcgctgggcgcccggcgcgccgctgagcgacgagcagacgcggttctacgacaccaacggctatctcgtgctggagaacgtgttcgaccccgccgagatcgcgctgctgcagtcggggtcgatggatctgctggccaaccccgccgggctcgaccgcgagaccatcatcaccgagcgcggcagcgacgaggtgcgctcgatcttcgcgatccacgcgcagaacgaattgctcggccgtctcgccgcggattcgcggattgccggggtggcgcgcttcctgctggatgacgacgtctacatccatcagtcgcggctcaactacaagccgggcttcgatggcaaggagttctactggcactccgatttcgagacctggcatgtcgaggatggcatgccgcggatgcgcgcgttgtcgatgtcgatcctgctggcggagaataccgcgaataacgggccgctgatggtcatccccggctcgcaccgcaaatatctcacctgcgttggcgagacgccggagaaccattaccgctcctcgctgaagaagcaggaatacggcgtgcccgaccgcgagatgctgaccgcgctcgccagcgatcacggcatcgtcgcgccgacgggcaaggccggcaccgtggtgctgttcgactgcaacacgatgcacggctcgaacggcaacatcacgccgttcccgcgctcgaacgcgttcttcgtgttcaacgcgaaggcgaacagcctggtcgagccgttcggcccgaaatcgcggcggccggacttcatcgccgaccgcgcgttcacgaccgtcgacatcgtgaagggcccgctggtgcggcgcgagcgcgcggcatga

SEQ ID NO: 20 - DNA, 921 bp, synthetic construct
  source 1..921: mol_type = other DNA
atggatgatttgtacccatcccgccgcgagccaaccccatccttgctcccacgtcacgacccagttgtccacggccgctgggctccaggtgcaccactctccgacgaacagacccgcttctacgataccaacggctacctggtgctcgagaacgtcttcgatccagccgaaatcgctctgctccagtccggctccatggacctgctcgcaaacccagccggcctggatcgcgaaaccatcatcaccgagcgcggctccgatgaagtgcgttccatcttcgctatccacgcacagaacgaattgctgggccgcctggcagctgattcccgcatcgccggcgtggctcgcttcctgctcgatgacgatgtctacatccaccagtcccgcctcaactacaagccaggcttcgatggcaaggagttctactggcactccgacttcgagacctggcacgtcgaagatggcatgccacgcatgcgcgcactgtccatgtccatcctgctcgctgaaaacaccgcaaacaacggcccactgatggtgatcccaggctcccaccgcaagtacctcacctgcgtcggcgaaaccccagagaaccactaccgctcctccctgaagaagcaggagtacggcgtgccagaccgcgaaatgctgaccgccctcgcttccgatcacggtatcgtggcaccaaccggcaaggctggtaccgtggtcctcttcgactgcaacaccatgcacggctccaacggcaacatcaccccattcccacgctccaacgccttcttcgtgttcaacgcaaaggccaactccctggtcgagccattcggtccaaagtcccgccgcccagacttcatcgcagatcgcgccttcaccaccgtggacatcgtgaagggtccactggtgcgtcgcgaacgtgctgcataa

SEQ ID NO: 21 - DNA, 936 bp, Alkalihalobacillus clausii
  source 1..936: mol_type = unassigned DNA
atgcaagaaaaggtagatctctatccttcacgcgttaaggagaccgcaaccataacggaaagaaaagatccaatcgtttattcaagggaaaaaggaccgctcgatcgtgaggaagtggctttttatgaggcaaatgggtatgtaatgttagaacggctttttcaagaagacgaagtgcaaatcatggctaatcaattggaagaggtgatgaaacagaaccaagagcgggacagtgatgaagtcatcaaagagcctgatagcaatgaaattcgctccgtttttgaagtccacaaagacaacggcttttttgaaatgttgtctaaacatgagcgcattgtggccattgcagaacaattgctaggcagccacgtgtacatcaaccaatcgcgcattaattttaaacctggctttaagggcaaagagtttttctggcattctgattttgaaacgtggcatgtggaagatgggatgccaaacatgcgggctgtcagctgctcgattatacttacggataactatgaatttaacgggcctttaatgcttatcccaggctcacataaatggtatgtttcttgtgcgggcacaacgccagacaaccattacaaatcatcgttaaagcaacaagttgcgggaacgcctgaccatacaagtttgcaatggctgactgaacaagcgggcggacggattgaccgtgctactggcccagccggatcggtgctgttttttgagtgcaatacgatgcatggctccaatgccaacctttctccttacccacgaagcaacgtctttttcgtatttaactcaattgaaaaccagttgcaggcaccttactcaggaaaacaaccaaggcctgaatttttagccaaccgcgacagcattgccccaattcaacctgtaaaagaaagcattgcccaacatgtccacgcaacgaaataa

SEQ ID NO: 22 - DNA, 936 bp, synthetic construct
  source 1..936: mol_type = other DNA
atgcaggaaaaggtggacctgtacccatcccgcgtcaaggaaaccgccaccatcaccgaacgcaaggacccaatcgtgtactcccgcgagaagggtccactggaccgtgaagaggtggctttctacgaagcaaacggctacgtcatgctggagcgcctcttccaggaagatgaggtgcagatcatggcaaaccagctggaagaggtcatgaagcagaaccaggaacgcgattccgacgaagtcatcaaggagccagattccaacgaaatccgctccgtgttcgaggtccacaaggacaacggcttcttcgaaatgctgtccaagcacgagcgcatcgtggcaatcgccgaacagctgctcggctcccacgtctacatcaaccagtcccgcatcaacttcaagccaggcttcaagggcaaggagttcttctggcactccgatttcgaaacctggcacgtggaggacggcatgccaaacatgcgcgctgtctcctgctccatcatcctgaccgacaactacgaattcaacggcccactgatgctcatcccaggctcccacaagtggtacgtgtcctgcgcaggcaccaccccagataaccactacaagtcctccctgaagcagcaggtggctggtaccccagaccacacctctttgcagtggctgaccgaacaggctggcggccgtatcgatcgtgcaaccggcccagctggctccgtgctgttcttcgagtgcaacaccatgcacggctccaacgcaaacctctccccatacccacgctccaacgtgttcttcgtcttcaactccatcgaaaaccagctgcaggcaccatactccggcaagcagccacgtccagagttcctcgctaaccgcgattccatcgcaccaatccagccagtgaaggaatccatcgcacagcacgtccacgccaccaagtaa

SEQ ID NO: 23 - DNA, 951 bp, Hydrocarboniclastica marina
  source 1..951: mol_type = unassigned DNA
atgctacagcgtacagacttttatccatccagactggattcgccggccgacagacttcgtcgcacagcacccaccgttcacgctcaaggtccgaaacgatggcagggtccgctggatgaacagagcctggcccgtttcgagcgagacggttttctctggttcgatggtttcttctcccgcgaccgggtcacgccgtttctggatgagcttcaggagctggcgaaggacactgccctggcaaattcagaacaggtcatcaaagacccgcaaagtggcgatctacgctcagttttcgctatgcacgagctctccgagcgcttcgaccagctgacccgggacccacgaatactgggtatggtgcagcagctcctcggcggggatgtctacatccatcagtcccgtataaacagtaaaaccggctttgcgggtagcggtttcgagtggcattcagactttgaaacctggcatgcagaggacggcatgccagaaatgcgagcagtgagcgcgtcactgatgctgacggacaacagtcccttcaatggcccgctcatgctcatacccggctcccacgattatttcgtgccttgcgtcggccgcacgcccgcggataactggaaacaatcgctgaaggatcagagcattggtgttcccgaccgcagccatattgcagctctggctgagcgcggcggaatcgaggcacctaccggaccagcaggctctctgctgttgttcgaatgcaacaccctgcatgcctcaaacagcaacatgtcaccctggccccgggctaacctgttcttcgtctacaacagtgtcgagaatcaactggtcgagcccttcagcggatcggcagcacgtcctgagtttctgggcgcgcgtaaaaacgtcaagccgttgaccatgcaagaacgccatgtcgaggccgatgaaactcagcacgtctacagcaactag

SEQ ID NO: 24 - DNA, 951 bp, synthetic construct
  source 1..951: mol_type = other DNA
atgctccagcgcaccgacttctacccatcccgcctggattccccagctgaccgtctccgtcgcaccgctccaaccgtgcacgcacagggtccaaagcgttggcagggtccactggatgagcagtccctcgcacgcttcgaacgcgatggcttcctgtggttcgacggcttcttctcccgcgatcgcgtcaccccattcctcgacgaactgcaggagctcgctaaggataccgccctcgctaactccgagcaggtgatcaaggacccacagtccggtgacctgcgctccgtcttcgcaatgcacgaactgtccgagcgcttcgatcagctgacccgcgacccacgcatcctgggtatggtgcagcagctgctcggcggcgacgtctacatccaccagtcccgcatcaactccaagaccggcttcgctggctccggcttcgaatggcactccgacttcgaaacctggcacgcagaggatggcatgccagaaatgcgcgcagtgtccgcctccctcatgctgaccgataactccccattcaacggcccactcatgctgatcccaggctcccacgactacttcgtgccatgcgtgggtcgtaccccagcagataactggaagcagtccctcaaggaccagtccatcggcgtgccagatcgttcccacatcgcagcactggctgaacgcggtggcatcgaagctccaaccggtccagctggctccctgctcctgttcgaatgcaacaccctgcacgcatccaactccaacatgtccccatggccacgcgccaacctcttcttcgtgtacaactccgtcgagaaccagctcgtggaaccattctccggctccgctgctcgcccagagttcctgggtgctcgtaagaacgtcaagccactgaccatgcaggaacgccacgtggaagctgatgagacccagcacgtctactccaactaa

SEQ ID NO: 25 - DNA, 960 bp, Methylomicrobium alcaliphilum
  source 1..960: mol_type = unassigned DNA
atgattaccgagaatgccgcacagtccgaacaaagtgaagatttttatcaatcacgtaacggtagtaagccgaaaataattccgcgcgtagacccggtagtttatgcgcaaacagctaatccaggtctcattgcagaggacttgcaagcacgttatgagcaacaaggttttcttgttattgataatgtttttaatgagagggaggtcgactgtttcaagcaagagctcaaacgcttgaacgacgatgaaaagataaaagcctcggcggaagcgataactgaattatccagcgacgaactccgttcactatttaaaattcatgaagtcagtccggtttttaaaaggttagctgccgataatcgattagcgggactggctcaacatcttttgaacgaccgggtttatattcatcagtcgcgcttaaactataagccgggttttcgcggcaaggaattttactggcattcggactttgaaacttggcatgtagaagacggtatgcctagaatgcgtgcgctcagcatgtccattattcttaccgaaaacgatcagcataacgggcctttgatgttggttcccggatcgcataaaaaatttgtcgtttgcgaagaggaaacgccggaaaatcattattcggtctcgttgaaaaagcaggagtacggcatacccagcgatgaatgcttggctagcttggttgccgatggcggcatcgtatcggccaatggaaaacccggcagtgtcttgattttcgacagtaatgtcatgcacggttcgaatagtaatatcactccatggcctcgctcgaatctctttttcgtctataacgcgatcaataatcgagtaacatggccgttttgcggtttattgccgcgtcctgaatatctttgcagtcgcaagaatatacgagttatcgaaccgcggccttttatcgcggccgccgatcaattgatatatgcttag

SEQ ID NO: 26 - DNA, 960 bp, synthetic construct
  source 1..960: mol_type = other DNA
atgatcaccgaaaacgcagcccagtccgagcagtccgaagatttctaccagtcccgcaacggctccaagccaaagatcatcccacgcgtggacccagtggtctacgcccagaccgctaacccaggcctgatcgccgaggatctgcaggctcgctacgaacagcagggcttcctggtgatcgataacgtcttcaacgagcgcgaagtggattgcttcaagcaggagctgaagcgcctcaacgatgacgaaaagatcaaggcctccgctgaggcaatcaccgaactgtcctccgacgagctgcgctccctcttcaagatccacgaagtgtccccagtcttcaagcgcctcgctgcagataaccgtctggcaggtctggcacagcacctgctcaacgaccgtgtgtacatccaccagtcccgcctgaactacaagccaggcttccgcggcaaggaattctactggcactccgatttcgagacctggcacgtcgaagacggcatgccacgcatgcgcgctctgtccatgtccatcatcctcaccgagaacgatcagcacaacggcccactgatgctcgtgccaggctcccacaagaagttcgtggtctgcgaagaggaaaccccagaaaaccactactccgtctccctgaagaagcaggagtacggcatcccatccgatgaatgcctggcttccctcgtggcagacggtggcatcgtctccgcaaacggcaagccaggctccgtgctgatcttcgattccaacgtcatgcacggctccaactccaacatcaccccatggccacgctccaacctcttcttcgtgtacaacgccatcaacaaccgcgtcacctggccattctgcggtctgctcccacgtccagagtacctgtgctcccgcaagaacatccgcgtgatcgaaccacgcccattcatcgccgctgcagaccagctcatctacgcctaa

SEQ ID NO: 27 - DNA, 894 bp, Neptunomonas concharum
  source 1..894: mol_type = unassigned DNA
atgcaagacgattacccctcacgcatagagaccagagccaaggtgcaaccgcgccttgatccggttatttatcctgaagcggaaacacccatactatcttcctgtacgttgtccacccagcaacttaacgattttgagaagaatggctaccttttgcttcccggactgtttaattcgtcggaggtcaatgagtttcaccaagccatcactgctatacagcaagatgagtctctcaaaaacagccctgttgccattaccgaaaggggcaattcagagctacgctctgttttccaaattcaccagaatcatccgctgttttcaaacgttgcccgcgacccacgcattgctgatattgcacggcgcattcttggcggtgatgtttatattcatcagtcacgtcttaacttcaagccaggctttaaaggcaaggagttttattggcactcggattttgaaacctggcatgtagaagatggcatgcctcgtatgcgagcaatcagctgctccattcttttgaccgataataatgcgaaaaatggcgctttaatgttgatgccaggctctcataaagagttcatcagttgcgttggcgaaacgcctgagaaccactacgagacatcattgcaaaagcaagaatatggcattcccagcaacgaaagcctgcaatacctaagcgataaatatggtattgattgcgcggaagccgccgcaggctctgtgctgttttttgattgcaacatcatgcatggttccaacagtaacattacgccggaccctcgcagcaacctattctttgtctacaaccatattgacaacatggtttatgagcctttttctctacaacctccacggccagaatatatctgctcgcgcgagaccataaaaaccctttaa

SEQ ID NO: 28 - DNA, 894 bp, synthetic construct
  source 1..894: mol_type = other DNA
atgcaggatgactacccatcccgcatcgaaacccgtgcaaaggtgcagccacgtctggacccagtcatctacccagaagccgagaccccaatcctctcctcctgcaccctgtccacccagcagctcaacgacttcgagaagaacggctacctgctcctgccaggcctcttcaactcctccgaagtcaacgagttccaccaggcaatcaccgccatccagcaggatgaatccctgaagaactccccagtggctatcaccgaacgtggtaactccgagctgcgctccgtcttccagatccaccagaaccacccactcttctccaacgtggcacgcgatccacgcatcgctgacatcgcacgccgcatcctgggcggcgatgtctacatccaccagtcccgcctcaacttcaagccaggcttcaagggcaaggagttctactggcactccgatttcgaaacctggcacgtggaggatggtatgccacgtatgcgtgccatctcctgctccatcctcctgaccgacaacaacgccaagaacggcgctctcatgctgatgccaggctcccacaaggaattcatctcctgcgtcggcgaaaccccagagaaccactacgaaacctctctccagaagcaggagtacggcatcccatccaacgaatccctccagtacctgtccgataagtacggtatcgactgcgcagaggcagctgctggctccgtgctgttcttcgactgcaacatcatgcacggctccaactccaacatcaccccagatccacgctccaacctgttcttcgtgtacaaccacatcgacaacatggtctacgaaccattctccctccagccaccacgcccagaatacatctgctcccgcgagaccatcaagaccctgtaa

SEQ ID NO: 29 - DNA, 918 bp, Leptospirillum ferriphilum
  source 1..918: mol_type = unassigned DNA
atgccatttcgactggaagaccgctacccgacccgcaaaaaccctgaacctgtctggatggagaggccggttcccgtgctgtatccgggacaccggaccccctctcccctttccgccgagcaggccggtcagtttgaccgggacggattcctcgtgttgccccggatctactcggatgaggaagtgcgggtcttccgggaggaggtcgagcgtttaagattggatccggaggtcagggcttcggaaaaaaccatccgggaaccccagggagacgctgtgcgttcggtgttcgcgatacaccgcgacaatcctctgtttgcccgcgtggcagcggatgagagaatcgcgggagtcgcgcgcttcctcctgggaggagacgtctatatccaccagtcccgcctgaactacaaaccgggattcaagggaaaagagttttactggcactcggatttcgagacatggcatgcggaagacggcatgcccgacatgcgggcggtaagctgttccatcctcctgaccgacaacaccacctctaacggccccctgatgctgattcccggctcccatcgccacttcatccattgcgtcgggcagacccccgagaaccattaccgggaatccctccgaaaacaggagtacggcgttccggaccaggcaagcctcgaaaaactcgccgctctttatggaatcacggaagtgacggcaccggcggggagcgcggttttcttcgactgcaacatcatgcacggctccaacagcaacatcaccccttttccgcgcacaaatcttttttatgtctacaaccatacggggaatgccgtgcaggaaggacttcggacgcaccctccgagaccggatttcgtcgccgaatccaaaaacttcactcctctcgcgattcgtccggagcgctttgcctga

SEQ ID NO: 30 - DNA, 918 bp, synthetic construct
  source 1..918: mol_type = other DNA
atgccattccgcctggaagatcgctacccaacccgcaagaacccagaaccagtctggatggagcgcccagttccagtgctgtacccaggtcaccgtaccccatccccactgtccgcagaacaggccggccagttcgatcgcgacggcttcctggtgctcccacgcatctactccgatgaagaggtgcgcgtcttccgtgaagaggtggaacgcctgcgtctcgacccagaagtccgtgcttccgagaagaccatccgtgaaccacagggtgatgctgtgcgctccgtcttcgctatccaccgcgataacccactcttcgcacgtgttgcagctgatgaacgtatcgctggcgtcgcacgcttcctgctcggcggcgacgtgtacatccaccagtcccgcctgaactacaagccaggcttcaagggcaaggagttctactggcactccgatttcgagacctggcacgctgaagatggcatgccagacatgcgcgcagtctcctgctccatcctgctcaccgacaacaccacctctaacggcccactgatgctcatcccaggctcccaccgccacttcatccactgcgtcggccagaccccagagaaccactaccgcgaatccctccgcaagcaggagtacggcgtgccagatcaggcatccctggaaaagctcgctgcactgtacggtatcaccgaggtgaccgcaccagctggctccgcagtcttcttcgactgcaacatcatgcacggctccaactccaacatcaccccattcccacgcaccaacctcttctacgtgtacaaccacaccggtaacgctgtccaggaaggcctgcgtacccacccaccacgcccagacttcgtggctgaatccaagaacttcaccccactggcaatccgcccagagcgcttcgcctaa

SEQ ID NO: 31 - DNA, 921 bp, Candidatus Nitrosopumilus sp.
  source 1..921: mol_type = unassigned DNA
atggctgaaaataagttttatttggattcttatcctacacgaacaagttctgaatcaaaaattattcaaagaacgaactctgttgtatattgtgattcttatgatgaattaaataaagaacaagtagatttttttgaaaaaaatggttatctaatatttgaaaatttattttcttctgatgagataactaaactgtttgatgagcttacctctctttcacaagatgaaataaaaaaagatcttcctcaattcattttagaagaaacacaaagagatgtacgttctatttttgaaattcataaaattagtaaactatatggcaaactttgtagagataagagaattttaaaaatagcacaacaacttttgggaagtaaggtctacattcatcaatcccgtgtaaaccttaaacctggatttgatggtaaagaattctattggcattctgattttgaaacatggcactctgaggatggtatgccaaacatgcgtgctgtttcatgttcaattagtttgactaaaaattatgaatttaatggacccttgatggtaatccctggttcacataaggaatttgtatcttgcagtgggaaaacacctgatgaacactataagcaatctctaaaaagacaggaaataggcactcctcaaaaagaatttctagaacaaatggttgaaaaaagtaagattgtatctgcaaaaggagatgcaggttcagtaatcttttttgattgtaatattatgcatggttcaaacggcaatatcacgccttatcctagaagtaatgccttttttgtttataatagcatccataataccttggttgatccattttgtggtttaaatcccagacctacctatattgcagaaagagaatttttgcctcttgagcctgttgataattttcttgattcaaaatag

SEQ ID NO: 32 - DNA, 921 bp, synthetic construct
  source 1..921: mol_type = other DNA
atggcagagaacaagttctacctggattcctaccctacccgcacctcttccgaatccaagatcatccagcgcaccaactccgtggtctactgcgattcctacgacgaactgaacaaggagcaggtggacttcttcgaaaagaacggctacctgatcttcgaaaacctcttctcctccgatgagatcaccaagctcttcgacgaactgacctctctctcccaggatgagatcaagaaggacctgccacagttcatcctcgaagagacccagcgcgatgtccgctccatcttcgaaatccacaagatctccaagctgtacggcaagctctgccgcgacaagcgcatcctgaagatcgcccagcagctgctcggctccaaggtgtacatccaccagtcccgcgtcaacctcaagccaggcttcgatggcaaggaattctactggcactccgatttcgaaacctggcactccgaggacggcatgccaaacatgcgcgctgtgtcctgctccatctccctgaccaagaactacgagttcaacggcccactcatggtgatcccaggctcccacaaggaattcgtctcctgctccggcaagaccccagacgagcactacaagcagtccctgaagcgccaggaaatcggcaccccacagaaggaattcctcgagcagatggtggagaagtccaagatcgtctccgcaaagggcgatgccggctccgtgatcttcttcgactgcaacatcatgcacggctccaacggcaacatcaccccatacccacgctccaacgctttcttcgtgtacaactccatccacaacaccctggtcgatccattctgcggcctcaacccacgcccaacctacatcgcagaacgcgagttcctgccactcgaaccagtcgataacttcctggactccaagtaa

SEQ ID NO: 33 - DNA, 921 bp, Sphyngopyxis alaskensis
  source 1..921: mol_type = unassigned DNA
atgcaagacctctacccctcgcgccagcgcgcggacgccgaaatgcggccgcggctggaccccgtcgtccatagcgaatggacaaacgatgcgccgatcagcgcgcggcaggccgcggcgttcgaccgcgacggctatatcgtgctcgaggatattttctcggccgacgaagtcgccttcctgcaaaaggccgcgggcaatctgctcgccgatccggcggcgctcgacgccgacacgatcgtcaccgagccgcaaagcaacgagatccgctcgatcttcgagattcacgcgcaaagcccggtgatggcgcgccttgccgccgatgcgcggctcgccgatgtcgcgcgcttcctgctcggcgacgaggtttatatccaccagtcgcggctgaactataaacccggtttcaagggcagggagttctactggcacagcgatttcgaaacctggcatgtcgaggacgggatgccgcggatgcgcgcgctgtcgatgtcggtgctgctcgccgaaaacaccccgcacaacggcccgctgatggtgattccgggctcgcaccgcacctatctcacctgcgtcggcgaaacccccgacgaccattatttaagctcgctcaagaaacaggaatatggcgtgcccgacgaggaaagcctcgccgaactggcgcacaggcacggcatcgtcgcgccgacgggcaagccgggaacggtgatcctgttcgactgcaatttgatgcacgggtcgaacggcaacatcacgccctttccgcgcgccaacgccttcctcgtctataatgccgtgagcaaccggctcgaaaagcccttcggcgtcgaaaagccgcgcccctggttcctcgcccgtcgcggcgagcccgcggcgctccgggttgagcgcgggccgctcgtcgaaacggtgccggcatga

SEQ ID NO: 34 - DNA, 921 bp, synthetic construct
  source 1..921: mol_type = other DNA
atgcaggatctgtacccatcccgccagcgcgctgatgcagaaatgcgtccacgtctcgacccagtggtccactccgagtggaccaacgatgctccaatctccgcacgtcaggcagcagctttcgatcgtgatggttacatcgtgctggaagacatcttctccgccgacgaggtcgctttcctccagaaggcagccggcaacctgctcgctgatccagctgcactggatgcagacaccatcgtgaccgaaccacagtccaacgagatccgctccatcttcgaaatccacgcacagtccccagtcatggcacgtctggctgctgatgctcgcctggctgatgtggctcgcttcctgctcggcgatgaagtctacatccaccagtcccgcctgaactacaagccaggcttcaagggccgcgagttctactggcactccgatttcgaaacctggcacgtggaagatggtatgccacgtatgcgcgcactctccatgtccgtcctgctcgctgaaaacaccccacacaacggcccactgatggtgatcccaggctcccaccgtacctacctcacctgcgtgggcgagaccccagatgaccactacctgtcctccctcaagaagcaggaatacggcgtgccagatgaagaatccctggcagagctggcacaccgtcacggtatcgtggcaccaaccggcaagccaggcaccgtcatcctgttcgactgcaacctcatgcacggctccaacggcaacatcaccccattcccacgcgccaacgctttcctggtgtacaacgcagtctccaaccgcctcgaaaagccattcggcgtggagaagccacgcccatggttcttggcacgccgcggcgaaccagcagcattgcgtgtggagcgcggtccactcgtggagaccgtcccagcataa

SEQ ID NO: 35 - DNA, 909 bp, Paenibacillus lautus
  source 1..909: mol_type = unassigned DNA
atgagtaagaatcatgcgtcggcccttcaggaaaaagaaatggacgtctatccttcaagagtgcatgcggaaccccggatcttaaaaaggcaggatccggtcgtacattcggagtggacgccggatgcgcccctaacgcaggagcaatccgacttctacgagcgcaacggatatttatttctggaaggcttctttgatcgggaggagctttcgcgatatcaggaggaggcccgcaggctgcagataacggcgcgggaatcggagaaagatgaagtgatccgggagcccggcggagacgaagtgcggtcggtattcgcggtacatgagagcgacgaagtgttcaagaagctgtcccagcatcctagactcctggcgatcatggaatacctcttgggaagcgagacgtatatccatcaatcccgaattaattacaagccgggctttacgggcaaggagttctactggcactccgatttcgaaacgtggcatgtcgaggacggcatgccgcgcatgagagcgctaagctgttccattgccctggaggacaactatccatataacgggccgcttatggtggtgcccggatcgcataaggaattcgtcgcctgcatcggccaaaccccggaggatcatttcaaggattccctgcgcaagcaggagtacggcgttccggatcatgacagcctgacgcggatggtgaaggagggcggaattgacacgccggtcggcaacgcgggctcgatcgtgatttttgactgcaacattatgcacggctcgaacagcaacatcacaccgatgccgcgaagcaatatctttatggtctataacagcgtggagaacaaggtcaagcagccgtattcgggccagaagccgagaccggagtatatcgccacccgtgagtctctatga

SEQ ID NO: 36 - DNA, 909 bp, synthetic construct
  source 1..909: mol_type = other DNA
atgtccaagaaccacgcatccgccctgcaggaaaaggagatggatgtgtacccatcccgcgtccacgctgaaccacgcatcctgaagcgccaggacccagtggtccactccgagtggaccccagatgcaccactcacccaggaacagtccgacttctacgagcgcaacggctacctgttcctcgaaggcttcttcgatcgcgaagagctgtcccgctaccaggaagaggcccgccgcctccagatcaccgctcgtgaatccgagaaggatgaagtgatccgtgagccaggcggcgacgaagtgcgctccgtcttcgcagtgcacgaatccgacgaggtcttcaagaagctgtcccagcacccacgcctgctcgccatcatggaatacctgctcggctccgagacctacatccaccagtcccgcatcaactacaagccaggcttcaccggcaaggaattctactggcactccgatttcgaaacctggcacgtggaggatggtatgccacgtatgcgtgctctgtcctgctccatcgcactcgaggataactacccatacaacggcccactcatggtggtcccaggctcccacaaggaattcgtggcctgcatcggccagaccccagaggatcacttcaaggactccctgcgcaagcaggaatacggcgtgccagatcacgactccctcacccgcatggtcaaggaaggcggcatcgataccccagtgggcaacgctggctccatcgtcatcttcgactgcaacatcatgcacggctccaactccaacatcaccccaatgccacgctccaacatcttcatggtctacaactccgtggaaaacaaggtcaagcagccatactccggccagaagccacgcccagaatacatcgcaacccgcgagtccctgtaa

SEQ ID NO: 37 - DNA, 999 bp, Chromohalobacter salexigens
  source 1..999: mol_type = unassigned DNA
atggcagtgtttgtcggcgccgacctctccgactacgttttctcggggatcggcggcaataccgttcccagcagactaatggaggagtttgcaatgaaagagacacaagacctgtttccgacgcgcctggaacgcaaactgggaatgttcgagcgcatcgatccggtcgtacacagtgaaggcgatcagcgcaaggggccgctcagcgaagccgagctcgacgagttcgaccgcaaggggttcctgtctttcgaggggttcttcgacgaggacgaaatggaagcgttcctccaggagctccgcgactacgagagcgatgaagacctcaagctctcggaaggcaccattctcgagcccggcaagcaggaaatccgttcgatcttcggcatccacgaggtgtcagaacgtttcagtcgtctgacgcgcgatccacgcctattggccatggtgcaacagatcctcggtggcgatgcctacattcaccaatcgcggatcaactacaagccgggcttcaagggcaagggcttcgactggcattcggatttcgagacctggcacagcgaggacggcatgccgcgcatgcgctcggtgagctgctcgatcattctcaccgaaaacggcgagttcaacggtccgctgatgctggtgcccggttcgcaccattatttcgtgccctgcgtggggcgtacgccggaggacaactacaaggagtcgctgaagagtcaagacatcggcgtgccggacgatgccagcctgcgcgacctgatgctcaagggcgatatcgaagcccccaagggtcccgtcgggtcgctggtgatgttcgagtgcaacaccctgcacggctccaacatcaacatgtcgtgctggccgcgcagcaacctgttcttcgtctacaacagtgtcgagaacacgctgcacgacccgtattgcggcaaccgtccgcggcccgagttcctcgccaaccgcaaggactggcggccgctgacaccggccgagtaa

SEQ ID NO: 38 - DNA, 999 bp, synthetic construct
  source 1..999: mol_type = other DNA
atggcagtgttcgtcggcgccgatctgtccgactacgtgttctccggtatcggcggcaacaccgtcccatcccgcctgatggaagagttcgccatgaaggaaacccaggatctcttcccaacccgcctggaacgcaagctcggcatgttcgagcgcatcgatccagtggtgcactccgaaggtgaccagcgtaagggtccactgtccgaagctgagctcgatgaattcgaccgcaagggcttcctgtccttcgagggcttcttcgatgaagacgagatggaagcattcctgcaggaactccgcgactacgagtccgatgaagacctgaagctctccgagggcaccatcctcgaaccaggcaagcaggagatccgctccatcttcggcatccacgaggtgtccgaacgtttctcccgcctgacccgcgatccacgcctgctcgctatggtccagcagatcctcggcggcgacgcatacatccaccagtcccgcatcaactacaagccaggcttcaagggcaagggcttcgattggcactccgacttcgaaacctggcactccgaggatggcatgccacgcatgcgctccgtgtcctgctccatcatcctgaccgagaacggcgaattcaacggcccactgatgctcgtcccaggctcccaccactacttcgtgccatgcgtcggccgcaccccagaagataactacaaggagtccctgaagtcccaggacatcggcgtgccagatgacgcatccctccgcgatctgatgctcaagggcgacatcgaagctccaaagggtccagtgggctccctggtcatgttcgagtgcaacaccctccacggctccaacatcaacatgtcctgctggccacgctccaacctgttcttcgtgtacaactccgtcgaaaacaccctccacgatccatactgcggtaaccgcccacgtccagagttcctggcaaaccgtaaggactggcgtccactcaccccagctgaataa

SEQ ID NO: 39 - DNA, 40 bp, synthetic construct
  source 1..40: mol_type = other DNA
ggccccccctcgaggtcgactggccgttaccctgcgaatg

SEQ ID NO: 40 - DNA, 40 bp, synthetic construct
  source 1..40: mol_type = other DNA
gtgaactgggtggtggtcattgtatgtcctcctggacttc

SEQ ID NO: 41 - DNA, 40 bp, synthetic construct
  source 1..40: mol_type = other DNA
gaagtccaggaggacatacaatgaccaccacccagttcac

SEQ ID NO: 42 - DNA, 40 bp, synthetic construct
  source 1..40: mol_type = other DNA
tggccggctgggcctctagattaagtcactggggccacgc

SEQ ID NO: 43 - DNA, 40 bp, synthetic construct; identical to SEQ ID NO: 39
  source 1..40: mol_type = other DNA

SEQ ID NO: 44 - DNA, 40 bp, synthetic construct
  source 1..40: mol_type = other DNA
gatgggtacaggtcttccattgtatgtcctcctggacttc

SEQ ID NO: 45 - DNA, 40 bp, synthetic construct
  source 1..40: mol_type = other DNA
gaagtccaggaggacatacaatggaagacctgtacccatc

SEQ ID NO: 46 - DNA, 40 bp, synthetic construct
  source 1..40: mol_type = other DNA
tggccggctgggcctctagattagttcactgcggagtaca

SEQ ID NO: 47 - DNA, 40 bp, synthetic construct; identical to SEQ ID NO: 39
  source 1..40: mol_type = other DNA

SEQ ID NO: 48 - DNA, 40 bp, synthetic construct
  source 1..40: mol_type = other DNA
tcctggcgtggggttgccactgtatgtcctcctggacttc

SEQ ID NO: 49 - DNA, 40 bp, synthetic construct
  source 1..40: mol_type = other DNA
gaagtccaggaggacatacagtggcaaccccacgccagga

SEQ ID NO: 50 - DNA, 40 bp, synthetic construct
  source 1..40: mol_type = other DNA
tggccggctgggcctctagattacttcactggggtgaagt

SEQ ID NO: 51 - DNA, 40 bp, synthetic construct
  source 1..40: mol_type = other DNA
gggaacaaaagctgggtacctggccgttaccctgcgaatg

SEQ ID NO: 52 - DNA, 40 bp, synthetic construct
  source 1..40: mol_type = other DNA
gggtacagatctgcctgcattgtatgtcctcctggacttc

SEQ ID NO: 53 - DNA, 40 bp, synthetic construct
  source 1..40: mol_type = other DNA
gaagtccaggaggacatacaatgcaggcagatctgtaccc

SEQ ID NO: 54 - DNA, 40 bp, synthetic construct
  source 1..40: mol_type = other DNA
ggctgggcctctagagtcgattacaggtactgctgtgggc

SEQ ID NO: 55 - DNA, 40 bp, synthetic construct; identical to SEQ ID NO: 39
  source 1..40: mol_type = other DNA

SEQ ID NO: 56 - DNA, 40 bp, synthetic construct
  source 1..40: mol_type = other DNA
gaggaggtctgcacggacattgtatgtcctcctggacttc

SEQ ID NO: 57 - DNA, 40 bp, synthetic construct
  source 1..40: mol_type = other DNA
gaagtccaggaggacatacaatgtccgtgcagacctcctc

SEQ ID NO: 58 - DNA, 40 bp, synthetic construct
  source 1..40: mol_type = other DNA
tggccggctgggcctctagattagccgtctggggaccagg

SEQ ID NO: 59 - DNA, 40 bp, synthetic construct
  source 1..40: mol_type = other DNA
ctgacgtcgggcccggtacctggccgttaccctgcgaatg

SEQ ID NO: 60 - DNA, 40 bp, synthetic construct; identical to SEQ ID NO: 40
  source 1..40: mol_type = other DNA

SEQ ID NO: 61 - DNA, 40 bp, synthetic construct; identical to SEQ ID NO: 41
  source 1..40: mol_type = other DNA

SEQ ID NO: 62 - DNA, 40 bp, synthetic construct
  source 1..40: mol_type = other DNA
agaagagcatcgatgtcgacttaagtcactggggccacgc

SEQ ID NO: 63 - DNA, 40 bp, synthetic construct; identical to SEQ ID NO: 59
  source 1..40: mol_type = other DNA

SEQ ID NO: 64 - DNA, 40 bp, synthetic construct; identical to SEQ ID NO: 44
  source 1..40: mol_type = other DNA

SEQ ID NO: 65 - DNA, 40 bp, synthetic construct; identical to SEQ ID NO: 45
  source 1..40: mol_type = other DNA

SEQ ID NO: 66 - DNA, 40 bp, synthetic construct
  source 1..40: mol_type = other DNA
agaagagcatcgatgtcgacttagttcactgcggagtaca

SEQ ID NO: 67 - DNA, 40 bp, synthetic construct; identical to SEQ ID NO: 59
  source 1..40: mol_type = other DNA

SEQ ID NO: 68 - DNA, 40 bp, synthetic construct; identical to SEQ ID NO: 48
  source 1..40: mol_type = other DNA

SEQ ID NO: 69 - DNA, 40 bp, synthetic construct; identical to SEQ ID NO: 49
  source 1..40: mol_type = other DNA

SEQ ID NO: 70 - DNA, 40 bp, synthetic construct
  source 1..40: mol_type = other DNA
agaagagcatcgatgtcgacttacttcactggggtgaagt

SEQ ID NO: 71 - DNA, 40 bp, synthetic construct
  source 1..40: mol_type = other DNA
cctgacgtcgggcccggtactggccgttaccctgcgaatg

SEQ ID NO: 72 - DNA, 40 bp, synthetic construct; identical to SEQ ID NO: 52
  source 1..40: mol_type = other DNA

SEQ ID NO: 73 - DNA, 40 bp, synthetic construct; identical to SEQ ID NO: 53
  source 1..40: mol_type = other DNA

SEQ ID NO: 74 - DNA, 40 bp, synthetic construct
  source 1..40: mol_type = other DNA
cagaagagcatcgatgtcgattacaggtactgctgtgggc

SEQ ID NO: 75 - DNA, 40 bp, synthetic construct; identical to SEQ ID NO: 59
  source 1..40: mol_type = other DNA

SEQ ID NO: 76 - DNA, 40 bp, synthetic construct; identical to SEQ ID NO: 56
  source 1..40: mol_type = other DNA

SEQ ID NO: 77 - DNA, 40 bp, synthetic construct; identical to SEQ ID NO: 57
  source 1..40: mol_type = other DNA

SEQ ID NO: 78 - DNA, 40 bp, synthetic construct
  source 1..40: mol_type = other DNA
agaagagcatcgatgtcgacttagccgtctggggaccagg